European Patent Application EP 4 545 086 A1, published April 30, 2025. Title: INCRETIN ANALOG AND AN USE THEREOF. Applicant: SHANGHAI MINWEI BIOTECHNOLOGY CO.,LTD. The sequence listing filed with the application follows.

SEQUENCE LISTING (13 sequences)

SEQ ID NO: 1 - protein, 39 aa, synthetic construct
  SITE 2: note = Xaa=Aib
  SITE 16: note = Lys at position 16 is chemically modified by conjugation of the epsilon-amino group of the Lys side chain with (2-[2-(2-amino-ethoxy)-ethoxy]-acetyl)-(yGlu)- CO-(CH2)18-CO2H
HXQGTFTSDYSILLDKIAAQAFIEWLIAGGPSSGAPPPS

SEQ ID NO: 2 - protein, 39 aa, synthetic construct
  SITE 2: note = Xaa=Aib
  SITE 16: note = Lys at position 16 is chemically modified by conjugation of the epsilon-amino group of the Lys side chain with (2-[2-(2-amino-ethoxy)-ethoxy]-acetyl)-(yGlu)- CO-(CH2)18-CO2H
HXQGTFTSDYSILLDKKAAQAFIEWLIAGGPSSGAPPPS

SEQ ID NO: 3 - protein, 39 aa, synthetic construct; identical to SEQ ID NO: 2
  SITE 2: note = Xaa=Aib
  SITE 17: note = Lys at position 17 is chemically modified by conjugation of the epsilon-amino group of the Lys side chain with (2-[2-(2-amino-ethoxy)-ethoxy]-acetyl)-(yGlu)- CO-(CH2)18-CO2H

SEQ ID NO: 4 - protein, 39 aa, synthetic construct
  SITE 2: note = Xaa=Aib
  SITE 16: note = Lys at position 16 is chemically modified by conjugation of the epsilon-amino group of the Lys side chain with (2-[2-(2-amino-ethoxy)-ethoxy]-acetyl)-(yGlu)- CO-(CH2)18-CO2H
HXQGTFTSDYSILLDKQAAQAFIEWLIAGGPSSGAPPPS

SEQ ID NO: 5 - protein, 39 aa, synthetic construct
  SITE 2: note = Xaa=Aib
  SITE 16: note = Lys at position 16 is chemically modified by conjugation of the epsilon-amino group of the Lys side chain with (2-[2-(2-amino-ethoxy)-ethoxy]-acetyl)-(yGlu)- CO-(CH2)18-CO2H
YXQGTFTSDYSILLDKIAAQAFIEWLIAGGPSSGAPPPS

SEQ ID NO: 6 - protein, 39 aa, synthetic construct
  SITE 2: note = Xaa=Aib
  SITE 16: note = Lys at position 16 is chemically modified by conjugation of the epsilon-amino group of the Lys side chain with (2-[2-(2-amino-ethoxy)-ethoxy]-acetyl)-(yGlu)- CO-(CH2)18-CO2H
HXQGTFTSDYSILLDKIAAQAFIEYLLEGGPSSGAPPPS

SEQ ID NO: 7 - protein, 39 aa, synthetic construct
  SITE 2: note = Xaa=Aib
  SITE 1: note = Xaa=His or Tyr
  SITE 16: note = Xaa = Lys or modified Lys
  SITE 17: note = Xaa = Ile or Gln or Lys or modified Lys
  SITE 25: note = Xaa = Trp or Tyr
  SITE 27: note = Xaa = Ile or Leu
  SITE 28: note = Xaa = Ala or Glu
XXQGTFTSDYSILLDXXAAQAFIEXLXXGGPSSGAPPPS

SEQ ID NO: 8 - protein, 39 aa, synthetic construct; identical to SEQ ID NO: 1
  SITE 2: note = Xaa=Aib

SEQ ID NO: 9 - protein, 39 aa, synthetic construct; identical to SEQ ID NO: 2
  SITE 2: note = Xaa=Aib

SEQ ID NO: 10 - protein, 39 aa, synthetic construct; identical to SEQ ID NO: 4
  SITE 2: note = Xaa=Aib

SEQ ID NO: 11 - protein, 39 aa, synthetic construct; identical to SEQ ID NO: 4
  SITE 2: note = Xaa=Aib

SEQ ID NO: 12 - protein, 39 aa, synthetic construct; identical to SEQ ID NO: 6
  SITE 2: note = Xaa=Aib

SEQ ID NO: 13 - protein, 39 aa, synthetic construct
  SITE 2: note = Xaa=Aib
  SITE 16: note = Lys at position 16 is chemically modified by conjugation of the epsilon-amino group of the Lys side chain with (2-[2-(2-amino-ethoxy)-ethoxy]-acetyl)-(yGlu)- CO-(CH2)18-CO2H
  SITE 25: note = Xaa = Trp or Tyr
  SITE 27: note = Xaa = Ile or Leu
  SITE 28: note = Xaa = Ala or Glu
HXQGTFTSDYSILLDXIAAQAFIEXLXXGGPSSGAPPPS